European Patent Specification EP 3 999 119 B1, published September 11, 2024. Title: Modified AAV capsid proteins for treatment of arthritic disease. Applicant: MEIRAGTX UK II LIMITED Universität Heidelberg. The sequence listing filed with the application follows.

SEQUENCE LISTING (30 sequences)

SEQ ID NO: 1 - protein, 745 aa, Artificial Sequence
  AAV1 with insert P4
MAADGYLPDWLEDNLSEGIREWWDLKPGAPKPKANQQKQDDGRGLVLPGYKYLGPFNGLDKGEPVNAADAAALEHDKAYDQQLKAGDNPYLRYNHADAEFQERLQEDTSFGGNLGRAVFQAKKRVLEPLGLVEEGAKTAPGKKRPVEQSPQEPDSSSGIGKTGQQPAKKRLNFGQTGDSESVPDPQPLGEPPATPAAVGPTTMASGGGAPMADNNEGADGVGNASGNWHCDSTWLGDRVITTSTRTWALPTYNNHLYKQISSASTGASNDNHYFGYSTPWGYFDFNRFHCHFSPRDWQRLINNNWGFRPKRLNFKLFNIQVKEVTTNDGVTTIANNLTSTVQVFSDSEYQLPYVLGSAHQGCLPPFPADVFMIPQYGYLTLNNGSQAVGRSSFYCLEYFPSQMLRTGNNFTFSYTFEEVPFHSSYAHSQSLDRLMNPLIDQYLYYLNRTQNQSGSAQNKDLLFSRGSPAGMSVQPKNWLPGPCYRQQRVSKTKTDNNNSNFTWTGASKYNLNGRESIINPGTAMASHKDDEDKFFPMSGVMIFGKESAGASNTALDNVMITDEEEIKATNPVATERFGTVAVNFQSSGQSGNDVRSANAQAAGDVHAMGALPGMVWQDRDVYLQGPIWAKIPHTDGHFHPSPLMGGFGLKNPPPQILIKNTPVPANPPAEFSATKFASFITQYSTGQVSVEIEWELQKENSKRWNPEVQYTSNYAKSANVDFTVDNNGLYTEPRPIGTRYLTRPL

SEQ ID NO: 2 - protein, 746 aa, Artificial Sequence
  AAV2 with insert P2
MAADGYLPDWLEDTLSEGIRQWWKLKPGPPPPKPAERHKDDSRGLVLPGYKYLGPFNGLDKGEPVNEADAAALEHDKAYDRQLDSGDNPYLKYNHADAEFQERLKEDTSFGGNLGRAVFQAKKRVLEPLGLVEEPVKTAPGKKRPVEHSPVEPDSSSGTGKAGQQPARKRLNFGQTGDADSVPDPQPLGQPPAAPSGLGTNTMATGSGAPMADNNEGADGVGNSSGNWHCDSTWMGDRVITTSTRTWALPTYNNHLYKQISSQSGASNDNHYFGYSTPWGYFDFNRFHCHFSPRDWQRLINNNWGFRPKRLNFKLFNIQVKEVTQNDGTTTIANNLTSTVQVFTDSEYQLPYVLGSAHQGCLPPFPADVFMVPQYGYLTLNNGSQAVGRSSFYCLEYFPSQMLRTGNNFTFSYTFEDVPFHSSYAHSQSLDRLMNPLIDQYLYYLSRTNTPSGTTTQSRLQFSQAGASDIRDQSRNWLPGPCYRQQRVSKTSADNNNSEYSWTGATKYHLNGRDSLVNPGPAMASHKDDEEKFFPQSGVLIFGKQGSEKTNVDIEKVMITDEEEIRTTNPVATEQYGSVSTNLQQGQSGCDCRGDCFCAQAATADVNTQGVLPGMVWQDRDVYLQGPIWAKIPHTDGHFHPSPLMGGFGLKHPPPQILIKNTPVPANPSTTFSAAKFASFITQYSTGQVSVEIEWELQKENSKRWNPEIQYTSNYNKSVNVDFTVDTNGVYSEPRPIGTRYLTRNL

SEQ ID NO: 3 - protein, 746 aa, Artificial Sequence
  AAV7 with insert A6
MAADGYLPDWLEDNLSEGIREWWDLKPGAPKPKANQQKQDNGRGLVLPGYKYLGPFNGLDKGEPVNAADAAALEHDKAYDQQLKAGDNPYLRYNHADAEFQERLQEDTSFGGNLGRAVFQAKKRVLEPLGLVEEGAKTAPAKKRPVEPSPQRSPDSSTGIGKKGQQPARKRLNFGQTGDSESVPDPQPLGEPPAAPSSVGSGTVAAGGGAPMADNNEGADGVGNASGNWHCDSTWLGDRVITTSTRTWALPTYNNHLYKQISSETAGSTNDNTYFGYSTPWGYFDFNRFHCHFSPRDWQRLINNNWGFRPKKLRFKLFNIQVKEVTTNDGVTTIANNLTSTIQVFSDSEYQLPYVLGSAHQGCLPPFPADVFMIPQYGYLTLNNGSQSVGRSSFYCLEYFPSQMLRTGNNFEFSYSFEDVPFHSSYAHSQSLDRLMNPLIDQYLYYLARTQSNPGGTAGNRELQFYQGGPSTMAEQAKNWLPGPCFRQQRVSKTLDQNNNSNFAWTGATKYHLNGRNSLVNPGVAMATHKDDEDRFFPSSGVLIFGKTGATNKTTLENVLMTNEEEIRPTNPVATEEYGIVSSNLQGQRGNEARVREAQAAQTQVVNNQGALPGMVWQNRDVYLQGPIWAKIPHTDGNFHPSPLMGGFGLKHPPPQILIKNTPVPANPPEVFTPAKFASFITQYSTGQVSVEIEWELQKENSKRWNPEIQYTSNFEKQTGVDFAVDSQGVYSEPRPIGTRYLTRNL

SEQ ID NO: 4 - protein, 745 aa, Artificial Sequence
  AAV9 with insert A2
MAADGYLPDWLEDNLSEGIREWWALKPGAPQPKANQQHQDNARGLVLPGYKYLGPGNGLDKGEPVNAADAAALEHDKAYDQQLKAGDNPYLKYNHADAEFQERLKEDTSFGGNLGRAVFQAKKRLLEPLGLVEEAAKTAPGKKRPVEQSPQEPDSSAGIGKSGAQPAKKRLNFGQTGDTESVPDPQPIGEPPAAPSGVGSLTMASGGGAPVADNNEGADGVGSSSGNWHCDSQWLGDRVITTSTRTWALPTYNNHLYKQISNSTSGGSSNDNAYFGYSTPWGYFDFNRFHCHFSPRDWQRLINNNWGFRPKRLNFKLFNIQVKEVTDNNGVKTIANNLTSTVQVFTDSDYQLPYVLGSAHEGCLPPFPADVFMIPQYGYLTLNDGSQAVGRSSFYCLEYFPSQMLRTGNNFQFSYEFENVPFHSSYAHSQSLDRLMNPLIDQYLYYLSKTINGSGQNQQTLKFSVAGPSNMAVQGRNYIPGPSYRQQRVSTTVTQNNNSEFAWPGASSWALNGRNSLMNPGPAMASHKEGEDRFFPLSGSLIFGKQGTGRDNVDADKVMITNEEEIKTTNPVATESYGQVATNHQGQRGNYSRGVDAQAAQTGWVQNQGILPGMVWQDRDVYLQGPIWAKIPHTDGNFHPSPLMGGFGMKHPPPQILIKNTPVPADPPTAFNKDKLNSFITQYSTGQVSVEIEWELQKENSKRWNPEIQYTSNYYKSNNVEFAVNTEGVYSEPRPIGTRYLTRNL

SEQ ID NO: 5 - protein, 747 aa, Artificial Sequence
  AAVrh10 with insert A6
MAADGYLPDWLEDNLSEGIREWWDLKPGAPKPKANQQKQDDGRGLVLPGYKYLGPFNGLDKGEPVNAADAAALEHDKAYDQQLKAGDNPYLRYNHADAEFQERLQEDTSFGGNLGRAVFQAKKRVLEPLGLVEEGAKTAPGKKRPVEPSPQRSPDSSTGIGKKGQQPAKKRLNFGQTGDSESVPDPQPIGEPPAGPSGLGSGTMAAGGGAPMADNNEGADGVGSSSGNWHCDSTWLGDRVITTSTRTWALPTYNNHLYKQISNGTSGGSTNDNTYFGYSTPWGYFDFNRFHCHFSPRDWQRLINNNWGFRPKRLNFKLFNIQVKEVTQNEGTKTIANNLTSTIQVFTDSEYQLPYVLGSAHQGCLPPFPADVFMIPQYGYLTLNNGSQAVGRSSFYCLEYFPSQMLRTGNNFEFSYQFEDVPFHSSYAHSQSLDRLMNPLIDQYLYYLSRTQSTGGTAGTQQLLFSQAGPNNMSAQAKNWLPGPCYRQQRVSTTLSQNNNSNFAWTGATKYHLNGRDSLVNPGVAMATHKDDEERFFPSSGVLMFGKQGAGKDNVDYSSVMLTSEEEIKTTNPVATEQYGVVADNLQGQRGNEARVREAQAAIVGAVNSQGALPGMVWQNRDVYLQGPIWAKIPHTDGNFHPSPLMGGFGLKHPPPQILIKNTPVPADPPTTFSQAKLASFITQYSTGQVSVEIEWELQKENSKRWNPEIQYTSNYYKSTNVDFAVNTDGTYSEPRPIGTRYLTRNL

SEQ ID NO: 6 - protein, 747 aa, Artificial Sequence
  AAVrh10 with insert A2
MAADGYLPDWLEDNLSEGIREWWDLKPGAPKPKANQQKQDDGRGLVLPGYKYLGPFNGLDKGEPVNAADAAALEHDKAYDQQLKAGDNPYLRYNHADAEFQERLQEDTSFGGNLGRAVFQAKKRVLEPLGLVEEGAKTAPGKKRPVEPSPQRSPDSSTGIGKKGQQPAKKRLNFGQTGDSESVPDPQPIGEPPAGPSGLGSGTMAAGGGAPMADNNEGADGVGSSSGNWHCDSTWLGDRVITTSTRTWALPTYNNHLYKQISNGTSGGSTNDNTYFGYSTPWGYFDFNRFHCHFSPRDWQRLINNNWGFRPKRLNFKLFNIQVKEVTQNEGTKTIANNLTSTIQVFTDSEYQLPYVLGSAHQGCLPPFPADVFMIPQYGYLTLNNGSQAVGRSSFYCLEYFPSQMLRTGNNFEFSYQFEDVPFHSSYAHSQSLDRLMNPLIDQYLYYLSRTQSTGGTAGTQQLLFSQAGPNNMSAQAKNWLPGPCYRQQRVSTTLSQNNNSNFAWTGATKYHLNGRDSLVNPGVAMATHKDDEERFFPSSGVLMFGKQGAGKDNVDYSSVMLTSEEEIKTTNPVATEQYGVVADNLQGQRGNYSRGVDAQAAIVGAVNSQGALPGMVWQNRDVYLQGPIWAKIPHTDGNFHPSPLMGGFGLKHPPPQILIKNTPVPADPPTTFSQAKLASFITQYSTGQVSVEIEWELQKENSKRWNPEIQYTSNYYKSTNVDFAVNTDGTYSEPRPIGTRYLTRNL

SEQ ID NO: 7 - protein, 748 aa, Artificial Sequence
  AAVDJ with insert QR-P2
MAADGYLPDWLEDTLSEGIRQWWKLKPGPPPPKPAERHKDDSRGLVLPGYKYLGPFNGLDKGEPVNEADAAALEHDKAYDRQLDSGDNPYLKYNHADAEFQERLKEDTSFGGNLGRAVFQAKKRLLEPLGLVEEAAKTAPGKKRPVEHSPVEPDSSSGTGKAGQQPARKRLNFGQTGDADSVPDPQPIGEPPAAPSGVGSLTMAAGGGAPMADNNEGADGVGNSSGNWHCDSTWMGDRVITTSTRTWALPTYNNHLYKQISNSTSGGSSNDNAYFGYSTPWGYFDFNRFHCHFSPRDWQRLINNNWGFRPKRLSFKLFNIQVKEVTQNEGTKTIANNLTSTIQVFTDSEYQLPYVLGSAHQGCLPPFPADVFMIPQYGYLTLNNGSQAVGRSSFYCLEYFPSQMLRTGNNFQFTYTFEDVPFHSSYAHSQSLDRLMNPLIDQYLYYLSRTQTTGGTTNTQTLGFSQGGPNTMANQAKNWLPGPCYRQQRVSKTSADNNNSEYSWTGATKYHLNGRDSLVNPGPAMASHKDDEEKFFPQSGVLIFGKQGSEKTNVDIEKVMITDEEEIRTTNPVATEQYGSVSTNLQQGQRGCDCRGDCFCAQAATADVNTQGVLPGMVWQDRDVYLQGPIWAKIPHTDGHFHPSPLMGGFGLKHPPPQILIKNTPVPADPPTTFNQSKLNSFITQYSTGQVSVEIEWELQKENSKRWNPEIQYTSNYYKSTSVDFAVNTEGVYSEPRPIGTRYLTRNL

SEQ ID NO: 8 - protein, 15 aa, Artificial Sequence
  insert A2
GQRGNYSRGVDAQAA

SEQ ID NO: 9 - protein, 15 aa, Artificial Sequence
  insert A6
GQRGNEARVREAQAA

SEQ ID NO: 10 - protein, 18 aa, Artificial Sequence
  insert P2
QGQSGCDCRGDCFCAQAA

SEQ ID NO: 11 - protein, 15 aa, Artificial Sequence
  insert P4
GQSGNDVRSANAQAA

SEQ ID NO: 12 - protein, 18 aa, Artificial Sequence
  insert QR-P2
QGQRGCDCRGDCFCAQAA

SEQ ID NO: 13 - protein, 736 aa, adeno-associated virus 1
MAADGYLPDWLEDNLSEGIREWWDLKPGAPKPKANQQKQDDGRGLVLPGYKYLGPFNGLDKGEPVNAADAAALEHDKAYDQQLKAGDNPYLRYNHADAEFQERLQEDTSFGGNLGRAVFQAKKRVLEPLGLVEEGAKTAPGKKRPVEQSPQEPDSSSGIGKTGQQPAKKRLNFGQTGDSESVPDPQPLGEPPATPAAVGPTTMASGGGAPMADNNEGADGVGNASGNWHCDSTWLGDRVITTSTRTWALPTYNNHLYKQISSASTGASNDNHYFGYSTPWGYFDFNRFHCHFSPRDWQRLINNNWGFRPKRLNFKLFNIQVKEVTTNDGVTTIANNLTSTVQVFSDSEYQLPYVLGSAHQGCLPPFPADVFMIPQYGYLTLNNGSQAVGRSSFYCLEYFPSQMLRTGNNFTFSYTFEEVPFHSSYAHSQSLDRLMNPLIDQYLYYLNRTQNQSGSAQNKDLLFSRGSPAGMSVQPKNWLPGPCYRQQRVSKTKTDNNNSNFTWTGASKYNLNGRESIINPGTAMASHKDDEDKFFPMSGVMIFGKESAGASNTALDNVMITDEEEIKATNPVATERFGTVAVNFQSSSTDPATGDVHAMGALPGMVWQDRDVYLQGPIWAKIPHTDGHFHPSPLMGGFGLKNPPPQILIKNTPVPANPPAEFSATKFASFITQYSTGQVSVEIEWELQKENSKRWNPEVQYTSNYAKSANVDFTVDNNGLYTEPRPIGTRYLTRPL

SEQ ID NO: 14 - protein, 735 aa, adeno-associated virus 2 [sequence omitted]

SEQ ID NO: 15 - protein, 737 aa, adeno-associated virus 7
MAADGYLPDWLEDNLSEGIREWWDLKPGAPKPKANQQKQDNGRGLVLPGYKYLGPFNGLDKGEPVNAADAAALEHDKAYDQQLKAGDNPYLRYNHADAEFQERLQEDTSFGGNLGRAVFQAKKRVLEPLGLVEEGAKTAPAKKRPVEPSPQRSPDSSTGIGKKGQQPARKRLNFGQTGDSESVPDPQPLGEPPAAPSSVGSGTVAAGGGAPMADNNEGADGVGNASGNWHCDSTWLGDRVITTSTRTWALPTYNNHLYKQISSETAGSTNDNTYFGYSTPWGYFDFNRFHCHFSPRDWQRLINNNWGFRPKKLRFKLFNIQVKEVTTNDGVTTIANNLTSTIQVFSDSEYQLPYVLGSAHQGCLPPFPADVFMIPQYGYLTLNNGSQSVGRSSFYCLEYFPSQMLRTGNNFEFSYSFEDVPFHSSYAHSQSLDRLMNPLIDQYLYYLARTQSNPGGTAGNRELQFYQGGPSTMAEQAKNWLPGPCFRQQRVSKTLDQNNNSNFAWTGATKYHLNGRNSLVNPGVAMATHKDDEDRFFPSSGVLIFGKTGATNKTTLENVLMTNEEEIRPTNPVATEEYGIVSSNLQAANTAAQTQVVNNQGALPGMVWQNRDVYLQGPIWAKIPHTDGNFHPSPLMGGFGLKHPPPQILIKNTPVPANPPEVFTPAKFASFITQYSTGQVSVEIEWELQKENSKRWNPEIQYTSNFEKQTGVDFAVDSQGVYSEPRPIGTRYLTRNL

SEQ ID NO: 16 - protein, 736 aa, adeno-associated virus 9
MAADGYLPDWLEDNLSEGIREWWALKPGAPQPKANQQHQDNARGLVLPGYKYLGPGNGLDKGEPVNAADAAALEHDKAYDQQLKAGDNPYLKYNHADAEFQERLKEDTSFGGNLGRAVFQAKKRLLEPLGLVEEAAKTAPGKKRPVEQSPQEPDSSAGIGKSGAQPAKKRLNFGQTGDTESVPDPQPIGEPPAAPSGVGSLTMASGGGAPVADNNEGADGVGSSSGNWHCDSQWLGDRVITTSTRTWALPTYNNHLYKQISNSTSGGSSNDNAYFGYSTPWGYFDFNRFHCHFSPRDWQRLINNNWGFRPKRLNFKLFNIQVKEVTDNNGVKTIANNLTSTVQVFTDSDYQLPYVLGSAHEGCLPPFPADVFMIPQYGYLTLNDGSQAVGRSSFYCLEYFPSQMLRTGNNFQFSYEFENVPFHSSYAHSQSLDRLMNPLIDQYLYYLSKTINGSGQNQQTLKFSVAGPSNMAVQGRNYIPGPSYRQQRVSTTVTQNNNSEFAWPGASSWALNGRNSLMNPGPAMASHKEGEDRFFPLSGSLIFGKQGTGRDNVDADKVMITNEEEIKTTNPVATESYGQVATNHQSAQAQAQTGWVQNQGILPGMVWQDRDVYLQGPIWAKIPHTDGNFHPSPLMGGFGMKHPPPQILIKNTPVPADPPTAFNKDKLNSFITQYSTGQVSVEIEWELQKENSKRWNPEIQYTSNYYKSNNVEFAVNTEGVYSEPRPIGTRYLTRNL

SEQ ID NO: 17 - protein, 738 aa, adeno-associated virus rh10
MAADGYLPDWLEDNLSEGIREWWDLKPGAPKPKANQQKQDDGRGLVLPGYKYLGPFNGLDKGEPVNAADAAALEHDKAYDQQLKAGDNPYLRYNHADAEFQERLQEDTSFGGNLGRAVFQAKKRVLEPLGLVEEGAKTAPGKKRPVEPSPQRSPDSSTGIGKKGQQPAKKRLNFGQTGDSESVPDPQPIGEPPAGPSGLGSGTMAAGGGAPMADNNEGADGVGSSSGNWHCDSTWLGDRVITTSTRTWALPTYNNHLYKQISNGTSGGSTNDNTYFGYSTPWGYFDFNRFHCHFSPRDWQRLINNNWGFRPKRLNFKLFNIQVKEVTQNEGTKTIANNLTSTIQVFTDSEYQLPYVLGSAHQGCLPPFPADVFMIPQYGYLTLNNGSQAVGRSSFYCLEYFPSQMLRTGNNFEFSYQFEDVPFHSSYAHSQSLDRLMNPLIDQYLYYLSRTQSTGGTAGTQQLLFSQAGPNNMSAQAKNWLPGPCYRQQRVSTTLSQNNNSNFAWTGATKYHLNGRDSLVNPGVAMATHKDDEERFFPSSGVLMFGKQGAGKDNVDYSSVMLTSEEEIKTTNPVATEQYGVVADNLQQQNAAPIVGAVNSQGALPGMVWQNRDVYLQGPIWAKIPHTDGNFHPSPLMGGFGLKHPPPQILIKNTPVPADPPTTFSQAKLASFITQYSTGQVSVEIEWELQKENSKRWNPEIQYTSNYYKSTNVDFAVNTDGTYSEPRPIGTRYLTRNL

SEQ ID NO: 18 - protein, 737 aa, Artificial Sequence
  AAV DJ-QR
MAADGYLPDWLEDTLSEGIRQWWKLKPGPPPPKPAERHKDDSRGLVLPGYKYLGPFNGLDKGEPVNEADAAALEHDKAYDRQLDSGDNPYLKYNHADAEFQERLKEDTSFGGNLGRAVFQAKKRLLEPLGLVEEAAKTAPGKKRPVEHSPVEPDSSSGTGKAGQQPARKRLNFGQTGDADSVPDPQPIGEPPAAPSGVGSLTMAAGGGAPMADNNEGADGVGNSSGNWHCDSTWMGDRVITTSTRTWALPTYNNHLYKQISNSTSGGSSNDNAYFGYSTPWGYFDFNRFHCHFSPRDWQRLINNNWGFRPKRLSFKLFNIQVKEVTQNEGTKTIANNLTSTIQVFTDSEYQLPYVLGSAHQGCLPPFPADVFMIPQYGYLTLNNGSQAVGRSSFYCLEYFPSQMLRTGNNFQFTYTFEDVPFHSSYAHSQSLDRLMNPLIDQYLYYLSRTQTTGGTTNTQTLGFSQGGPNTMANQAKNWLPGPCYRQQRVSKTSADNNNSEYSWTGATKYHLNGRDSLVNPGPAMASHKDDEEKFFPQSGVLIFGKQGSEKTNVDIEKVMITDEEEIRTTNPVATEQYGSVSTNLQRGNRQAATADVNTQGVLPGMVWQDRDVYLQGPIWAKIPHTDGHFHPSPLMGGFGLKHPPPQILIKNTPVPADPPTTFNQSKLNSFITQYSTGQVSVEIEWELQKENSKRWNPEIQYTSNYYKSTSVDFAVNTEGVYSEPRPIGTRYLTRNL

SEQ ID NO: 19 - protein, 724 aa, adeno-associated virus 5
MSFVDHPPDWLEEVGEGLREFLGLEAGPPKPKPNQQHQDQARGLVLPGYNYLGPGNGLDRGEPVNRADEVAREHDISYNEQLEAGDNPYLKYNHADAEFQEKLADDTSFGGNLGKAVFQAKKRVLEPFGLVEEGAKTAPTGKRIDDHFPKRKKARTEEDSKPSTSSDAEAGPSGSQQLQIPAQPASSLGADTMSAGGGGPLGDNNQGADGVGNASGDWHCDSTWMGDRVVTKSTRTWVLPSYNNHQYREIKSGSVDGSNANAYFGYSTPWGYFDFNRFHSHWSPRDWQRLINNYWGFRPRSLRVKIFNIQVKEVTVQDSTTTIANNLTSTVQVFTDDDYQLPYVVGNGTEGCLPAFPPQVFTLPQYGYATLNRDNTENPTERSSFFCLEYFPSKMLRTGNNFEFTYNFEEVPFHSSFAPSQNLFKLANPLVDQYLYRFVSTNNTGGVQFNKNLAGRYANTYKNWFPGPMGRTQGWNLGSGVNRASVSAFATTNRMELEGASYQVPPQPNGMTNNLQGSNTYALENTMIFNSQPANPGTTATYLEGNMLITSESETQPVNRVAYNVGGQMATNNQSSTTAPATGTYNLQEIVPGSVWMERDVYLQGPIWAKIPETGAHFHPSPAMGGFGLKHPPPMMLIKNTPVPGNITSFSDVPVSSFITQYSTGQVTVEMEWELKKENSKRWNPEIQYTNNYNDPQFVDFAPDSTGEYRTTRPIGTRYLTRPL

SEQ ID NO: 20 - protein, 13 aa, Artificial Sequence
  insertAAV7A6
GQRGNEARVREAQ

SEQ ID NO: 21 - protein, 15 aa, Artificial Sequence
  insertAAV2P2
QGQSGCDCRGDCFCA

SEQ ID NO: 22 - protein, 15 aa, Artificial Sequence
  insertAAVDJQRP2
QGQRGCDCRGDCFCA

SEQ ID NO: 23 - protein, 17 aa, Artificial Sequence
  general formula I
  MISC_FEATURE (1)..(1): Xaa represents 0, 1 or 2 amino acid residues
  MISC_FEATURE (4)..(4): Xaa represents a single amino acid residue
  MISC_FEATURE (6)..(6): Xaa represents a single amino acid residue
  MISC_FEATURE (7)..(7): Xaa represents a single amino acid residue
  MISC_FEATURE (8)..(8): Xaa represents a single amino acid residue
  MISC_FEATURE (10)..(10): Xaa represents a single amino acid residue
  MISC_FEATURE (11)..(11): Xaa represents a single amino acid residue
  MISC_FEATURE (12)..(12): Xaa represents a single amino acid residue
  MISC_FEATURE (13)..(13): Xaa represents 0, 1 or 2 amino acid residues
XGQXGXXXRXXXXAQAA

SEQ ID NO: 24 - protein, 19 aa, Artificial Sequence
  alternative formula for sequence Z
  MISC_FEATURE (1)..(1): Xaa is Q or none
  MISC_FEATURE (4)..(4): Xaa is S or R
  MISC_FEATURE (6)..(6): Xaa is N or C
  MISC_FEATURE (7)..(7): Xaa is D, Y or E
  MISC_FEATURE (8)..(8): Xaa is C, V, S or A
  MISC_FEATURE (10)..(10): Xaa is G, S or V
  MISC_FEATURE (11)..(11): Xaa is none, A, V or R
  MISC_FEATURE (12)..(12): Xaa is D, N or E
  MISC_FEATURE (13)..(13): Xaa is  C or A
  MISC_FEATURE (14)..(14): Xaa is  F or Q
  MISC_FEATURE (15)..(15): Xaa is  none, C or A
  MISC_FEATURE (16)..(16): Xaa is  none or A
  MISC_FEATURE (17)..(17): Xaa is none or Q
  MISC_FEATURE (18)..(18): Xaa is none or A
  MISC_FEATURE (19)..(19): Xaa is none or A
XGQXGXXXRXXXXXXXXXX

SEQ ID NO: 25 - protein, 18 aa, Artificial Sequence
  alternative formula for sequence Z
  MISC_FEATURE (1)..(1): Xaa is Q or none
  MISC_FEATURE (4)..(4): Xaa is S or R
  MISC_FEATURE (6)..(6): Xaa is N or C
  MISC_FEATURE (7)..(7): Xaa is D, Y or E
  MISC_FEATURE (8)..(8): Xaa is C, V, S or A
  MISC_FEATURE (10)..(10): Xaa is G, S or V
  MISC_FEATURE (11)..(11): Xaa is none or D
  MISC_FEATURE (12)..(12): Xaa is none or C
  MISC_FEATURE (13)..(13): Xaa is A, V, R or F
  MISC_FEATURE (14)..(14): Xaa is N, D, E or C
  MISC_FEATURE (16)..(16): Xaa is none or Q
  MISC_FEATURE (17)..(17): Xaa is none or A
  MISC_FEATURE (18)..(18): Xaa is none or A
XGQXGXXXRXXXXXAXXX

SEQ ID NO: 26 - protein, 18 aa, Artificial Sequence
  preferred embodiment of formula I
  MISC_FEATURE (1)..(1): Xaa is none or Q
  MISC_FEATURE (4)..(4): Xaa is R or S
  MISC_FEATURE (6)..(6): Xaa is C or N
  MISC_FEATURE (7)..(7): Xaa is D, E or Y
  MISC_FEATURE (8)..(8): Xaa is C, A, S or V
  MISC_FEATURE (10)..(10): Xaa is G, V or S
  MISC_FEATURE (11)..(11): Xaa is D or none
  MISC_FEATURE (12)..(12): Xaa is C or none
  MISC_FEATURE (13)..(13): Xaa is F, R, V or A
  MISC_FEATURE (14)..(14): Xaa is C, D, N or E
XGQXGXXXRXXXXXAQAA

SEQ ID NO: 27 - protein, 52 aa, Artificial Sequence
  formula II
  MISC_FEATURE (5)..(8): Xaa represents a single amino acid residue
  MISC_FEATURE (14)..(15): Xaa represents a single amino acid residue
  MISC_FEATURE (17)..(20): Xaa represents a single amino acid residue
  MISC_FEATURE (22)..(22): Xaa represents a single amino acid residue
  MISC_FEATURE (24)..(24): Xaa represents 0, 1 or 2 amino acid residue(s)
  MISC_FEATURE (25)..(25): Xaa represents sequence Z
  MISC_FEATURE (26)..(26): Xaa represents 5, 6, 7, 8, 9, 10, 11, 12, 13, 14 or 15 amino acid residues
  MISC_FEATURE (34)..(34): Xaa represents a single amino acid residue
EEEIXXXXPVATEXXGXXXXNXQXXXLPGMVWQXRDVYLQGPIWAKIPHTDG

SEQ ID NO: 28 - DNA, 1470 bp, artificial sequence
  etanercept
atggctcctgtcgccgtctgggccgcactggctgtcgggctggaactgtgggccgccgcacatgcactgcccgctcaggtcgcattcaccccatacgcacctgagccaggaagcacatgcaggctgagagagtactatgatcagaccgcccagatgtgctgttccaagtgctctcccggccagcacgccaaggtgttctgtaccaagacatccgacacagtgtgcgatagctgtgaggactccacctacacacagctgtggaactgggtgcctgagtgcctgagctgtggctcccggtgcagctccgaccaggtggagacacaggcctgtacacgggagcagaatagaatctgcacctgtaggcctggctggtattgcgcactgagcaagcaggagggatgcaggctgtgcgcaccactgaggaagtgtaggcctggattcggagtggccaggccaggcaccgagacaagcgatgtggtgtgcaagccctgtgcccctggcaccttttccaacaccacatctagcacagacatctgccgcccccaccagatctgtaacgtggtggccatccctggcaatgcctctatggatgccgtgtgcacctccacatctccaacccggagcatggcaccaggagcagtgcacctgccacagcccgtgagcacaagaagccagcacacccagccaacaccagagcctagcaccgcaccaagcacatccttcctgctgccaatgggaccatctccacctgcagagggaagcaccggcgatgagcctaagtcttgcgacaagacccacacatgcccaccatgtccagcaccagagctgctgggaggaccttccgtgttcctgtttcctccaaagccaaaggataccctgatgatctcccggacccctgaggtgacatgcgtggtggtggacgtgagccacgaggacccagaggtgaagtttaactggtacgtggacggcgtggaggtgcacaatgccaagaccaagcccagggaggagcagtacaactccacctatcgcgtggtgtctgtgctgacagtgctgcaccaggactggctgaacggcaaggagtataagtgcaaggtgagcaataaggccctgcctgccccaatcgagaagaccatctccaaggcaaagggacagcctagggagccacaggtgtacacactgcccccttccagagaggagatgaccaagaaccaggtgtctctgacatgtctggtgaagggcttctatccatctgatatcgccgtggagtgggagagcaatggccagcccgagaacaattacaagaccacaccacccgtgctggactccgatggctctttctttctgtatagcaagctgaccgtggacaagtccaggtggcagcagggcaacgtgttcagctgcagcgtgatgcacgaagcactgcacaatcattacacccagaagtcactgtcactgtctccagggaagtag

SEQ ID NO: 29 - protein, 489 aa, artificial sequence
  etanercept + signal peptide
MAPVAVWAALAVGLELWAAAHALPAQVAFTPYAPEPGSTCRLREYYDQTAQMCCSKCSPGQHAKVFCTKTSDTVCDSCEDSTYTQLWNWVPECLSCGSRCSSDQVETQACTREQNRICTCRPGWYCALSKQEGCRLCAPLRKCRPGFGVARPGTETSDVVCKPCAPGTFSNTTSSTDICRPHQICNVVAIPGNASMDAVCTSTSPTRSMAPGAVHLPQPVSTRSQHTQPTPEPSTAPSTSFLLPMGPSPPAEGSTGDEPKSCDKTHTCPPCPAPELLGGPSVFLFPPKPKDTLMISRTPEVTCVVVDVSHEDPEVKFNWYVDGVEVHNAKTKPREEQYNSTYRVVSVLTVLHQDWLNGKEYKCKVSNKALPAPIEKTISKAKGQPREPQVYTLPPSREEMTKNQVSLTCLVKGFYPSDIAVEWESNGQPENNYKTTPPVLDSDGSFFLYSKLTVDKSRWQQGNVFSCSVMHEALHNHYTQKSLSLSPGK

SEQ ID NO: 30 - protein, 467 aa, artificial sequence
  etanercept
LPAQVAFTPYAPEPGSTCRLREYYDQTAQMCCSKCSPGQHAKVFCTKTSDTVCDSCEDSTYTQLWNWVPECLSCGSRCSSDQVETQACTREQNRICTCRPGWYCALSKQEGCRLCAPLRKCRPGFGVARPGTETSDVVCKPCAPGTFSNTTSSTDICRPHQICNVVAIPGNASMDAVCTSTSPTRSMAPGAVHLPQPVSTRSQHTQPTPEPSTAPSTSFLLPMGPSPPAEGSTGDEPKSCDKTHTCPPCPAPELLGGPSVFLFPPKPKDTLMISRTPEVTCVVVDVSHEDPEVKFNWYVDGVEVHNAKTKPREEQYNSTYRVVSVLTVLHQDWLNGKEYKCKVSNKALPAPIEKTISKAKGQPREPQVYTLPPSREEMTKNQVSLTCLVKGFYPSDIAVEWESNGQPENNYKTTPPVLDSDGSFFLYSKLTVDKSRWQQGNVFSCSVMHEALHNHYTQKSLSLSPGK